European Patent Application EP 4 389 864 A1, published June 26, 2024. Title: Cutinases. Applicant: BASF SE. The sequence listing filed with the application follows.

SEQUENCE LISTING (10 sequences)

SEQ ID NO: 1 - DNA, 777 bp, synthetic construct
  source 1..777: mol_type = other DNA
gccgaaaatccgtacgaacggggtccggcccccacaacggcgtccattgaggcggcaaggggaccgtacgcgacatcgagtactaccgtatcgtcctttgcggcccggggatttgggggaggcacaatctattatcctacttcaacggcggatggaacgtttggagcagttgctgtgtccccaggatatacagcagcacaaagctcaatctcatggctgggcccgcgcttagcgagtcagggctttgttgtgttcaccattgacacgaatagcaggtacgaccagccgggtagcagagcggatcagttagcagcggctctcgactatcttactgaatcttcgacggtccgcagcagagttgatgcgtcgcgcctggctgtcatgggccattcaatgggcggtggcggcgccattgaagccgcttctgatgatccgtctcttaaggcagccgtggctttgacaccctggcacttgacgaaaacctggagccgcgtttcgacaccgacgatggtagtcggggcagaaaacgattctgtggccagcacacgttcccacgcggtcccgttgtattcaggaataccttcgtctaccccgaaggcctacctggagctccgaggcgccagccattttgcgcctaacaccagcaacacgacaatcgcaaaatacagcctggcttggcttaaacgctgggtcgatgacgacacgcgttatacgcaattcattgccccaggccctgggacgtcaacagctatctccgactggagacggtcagggtat

SEQ ID NO: 2 - protein, 259 aa, Pseudomonas mendocina (strain ymp)
AENPYERGPAPTTASIEAARGPYATSSTTVSSFAARGFGGGTIYYPTSTADGTFGAVAVSPGYTAAQSSISWLGPRLASQGFVVFTIDTNSRYDQPGSRADQLAAALDYLTESSTVRSRVDASRLAVMGHSMGGGGAIEAASDDPSLKAAVALTPWHLTKTWSRVSTPTMVVGAENDSVASTRSHAVPLYSGIPSSTPKAYLELRGASHFAPNTSNTTIAKYSLAWLKRWVDDDTRYTQFIAPGPGTSTAISDWRRSGY

SEQ ID NO: 3 - DNA, 777 bp, synthetic construct
  source 1..777: mol_type = other DNA
gccgacaacccatacgaacggggcccggaccccacagaatcaagtattgaagcatctcgcgggccgtttgcagtcagccagacgacagtcagctccctcgttgttagcggattcggaggcggcacgatctattatccgacggatacgagccagggaacgtttggagccgtggcgatttcgcctggctatacagcggatcaaacctcgattgcgtggattggaccgcggttggcctcgcagggattcgtggtctttacaatcgatacaatcacccgttacgatcagcccgcaagcagaggcgatcaattgcttgcggcgcttgattatctgacccagcgatcttccgtagcatcacgcattgactcgtcacggctaggagtcgcggggcactcaatgggcggggggggcacgctcgaggcggctgacgagcgcccgagccttcaagctgccgttccgctggccccgtggaatttgagaaaaaacttctcctcagtacaagtgccgacgtttatcatcggcggtgaatctgatacagtcgctccggttgcaacgcattcggaaccattttacacctccttaccttcttccctggataaagcttacatggaactgaataacgcctctcatttttttcctaatacatcaaatactacaatggccaaatatatgataagctggttcaagaggttcatcgacaacgacacgaggtatgatcaatttctttgtccgaaccctagtggtttagcaatcgaagagtatagaagcacttgcccttac

SEQ ID NO: 4 - protein, 259 aa, Amycolatopsis keratiniphila
ADNPYERGPDPTESSIEASRGPFAVSQTTVSSLVVSGFGGGTIYYPTDTSQGTFGAVAISPGYTADQTSIAWIGPRLASQGFVVFTIDTITRYDQPASRGDQLLAALDYLTQRSSVASRIDSSRLGVAGHSMGGGGTLEAADERPSLQAAVPLAPWNLRKNFSSVQVPTFIIGGESDTVAPVATHSEPFYTSLPSSLDKAYMELNNASHFFPNTSNTTMAKYMISWFKRFIDNDTRYDQFLCPNPSGLAIEEYRSTCPY

SEQ ID NO: 5 - DNA, 777 bp, synthetic construct
  source 1..777: mol_type = other DNA
gcagtctctccgtatcagcatggccctgatcccacagaggatttgattgaagcaccccgtggtccgtacgcgacggcccagatctcggtcagcaggctgagcgtgacgggctttggtggaggagtcatctattacccaacgacaacatcagaaggacgctttggcgcgatcgctattagcccgggctttacagcgacgtggtcatctctggactggctgggacctcggttggcgtcacacggattcgtggtttttggtatagaaacaaacacgctcctggatcagccggactcacgcggggcacaactgttagctgctttggactatcttacccaacgctcttccgtccgggatagagtagatgcgagccggctggcagtagcagggcattcaatggggggaggcgggacgttagaagccgccaaatccagaccgagtttgaaggctgccatccctattgccccgtggaatcttgacaagacctggccggaagtccgtacaccgacgctgatcatcggcggccaacttgatacgattgcccctgttgcaacccattccatcccgttctatctctccctttcgaacgcgcctgagaaaggctacctcgaattactaggagcctcgcactttttcccgcaaacgtctaacacaactatggcgaaatatatgattagctggatgaaacgcttcattgacgacgatacaaggtactcgcagtttctttgtccggcgccaaatgattttaccctcagcgatagcagagtgacttgccccgtt

SEQ ID NO: 6 - protein, 259 aa, Pseudomonas bauzanensis
AVSPYQHGPDPTEDLIEAPRGPYATAQISVSRLSVTGFGGGVIYYPTTTSEGRFGAIAISPGFTATWSSLDWLGPRLASHGFVVFGIETNTLLDQPDSRGAQLLAALDYLTQRSSVRDRVDASRLAVAGHSMGGGGTLEAAKSRPSLKAAIPIAPWNLDKTWPEVRTPTLIIGGQLDTIAPVATHSIPFYLSLSNAPEKGYLELLGASHFFPQTSNTTMAKYMISWMKRFIDDDTRYSQFLCPAPNDFTLSDSRVTCPV

SEQ ID NO: 7 - DNA, 768 bp, synthetic construct
  source 1..768: mol_type = other DNA
gcggttcatggaccggatccgacggacgctctgttagaggcctcgaggggcccctacgcgaccgcgcagattgacgtatcgtctctgtcggtgagcggctttggtgggggcacgatttattatccgacgacgacgtccgaaggcacatttggcggcgtcgcgatcgcacccggatatactgcagataaatcatcattagcctggcttgcagcgcgacttgcttctcacgggtttgtggtgtttaatatcgatacattaacaagactggaccaacctgacagccgcggtcgccaactgctggccgcacttgactatctcacgcagagatcatccgtccgcggccgggtcgatgccaccagattgggagtcatgggccatagcatgggcggaggcggtaccttggaagcggtagcagatcgtcctagtcttagggcggctgtcccgctgacaccgtggaacctcgataagacgtggtccggagtccagacacctacacttattataggagccgataacgacaccgtcgctccagttgccagccatgcagagccgttctatacgtcgttgccgagctcattggacaaagcgtacctcgaattgaataacgccacccacttcgccccaaacacaacgaatacaacaatcggaaaatacgcggttgcttggatgaagcggtttgttgatgatgatactcggtacggacgctttctctgcccggggcctagcagcgggctgcttgtggaagaatatcgttctacgtgtccgttc

SEQ ID NO: 8 - protein, 256 aa, Amycolatopsis orientalis HCCB10007
AVHGPDPTDALLEASRGPYATAQIDVSSLSVSGFGGGTIYYPTTTSEGTFGGVAIAPGYTADKSSLAWLAARLASHGFVVFNIDTLTRLDQPDSRGRQLLAALDYLTQRSSVRGRVDATRLGVMGHSMGGGGTLEAVADRPSLRAAVPLTPWNLDKTWSGVQTPTLIIGADNDTVAPVASHAEPFYTSLPSSLDKAYLELNNATHFAPNTTNTTIGKYAVAWMKRFVDDDTRYGRFLCPGPSSGLLVEEYRSTCPF

SEQ ID NO: 9 - DNA, 795 bp, synthetic construct
  source 1..795: mol_type = other DNA
gctccgctggccgataatccgtatgaacgcggcccggcaccaacaaccagcagcattgaagcgtccagaggatcgttcgcaacagcgacgacgaccgtgtccggcttgtctgtgacaggcttcggcggaggaacaatctactatccgacgagcacagctcagggaacctttggcgcagtcgctgtcgctccggggtttactgcatatcagtcctcaatggcctggcttgggccacgcttggcctcgcaaggctttgtggtattcacgatcgatacgaacacgacactagaccaaccggattctcgcggcaggcagctgctggcagcgcttgactacttaacagaaagatcgtccgttcgatcacggattgatagcagccggttaggtgtcataggccattccatgggaggcggtggaaccctcgaggcagcgcgctctagaccgacgctccaagccgccatcccgcttactgggtggaaccttacgaccaactggtcaggtaaccgtgtaccgacacttgtcgttggcgcgcagagcgacgccatcgcgcctgttggaagccacagtatccccttttataattcactcccctcgacattggataaagcctacttggagctgcgcggagccagtcatttcgctccgaatacggcgaatacaactattgcgaagtatacgattagctggctgaaacgttttatcgacaacgatacgcggtacgaacagtttttatgtcctatcccttcaaccaatctgcaaatttcggcgtttagggggaactgccctcactcatct

SEQ ID NO: 10 - protein, 265 aa, Pseudomonas sp. BICA1-14
APLADNPYERGPAPTTSSIEASRGSFATATTTVSGLSVTGFGGGTIYYPTSTAQGTFGAVAVAPGFTAYQSSMAWLGPRLASQGFVVFTIDTNTTLDQPDSRGRQLLAALDYLTERSSVRSRIDSSRLGVIGHSMGGGGTLEAARSRPTLQAAIPLTGWNLTTNWSGNRVPTLVVGAQSDAIAPVGSHSIPFYNSLPSTLDKAYLELRGASHFAPNTANTTIAKYTISWLKRFIDNDTRYEQFLCPIPSTNLQISAFRGNCPHSS